European Patent Application EP 4 631 966 A1, published October 15, 2025. Title: 신규한 펩타이드. Applicant: 하이센스바이오. Application KR, filed November 2, 2023. The sequence listing filed with the application follows.

SEQUENCE LISTING (64 sequences)

SEQ ID NO: 1 - protein, 10 aa, synthetic construct
KYKAKKKNYK

SEQ ID NO: 2 - protein, 10 aa, synthetic construct
KYKAKKRNYK

SEQ ID NO: 3 - protein, 10 aa, synthetic construct
KYKAKRKNYK

SEQ ID NO: 4 - protein, 10 aa, synthetic construct
KYKARKKNYK

SEQ ID NO: 5 - protein, 10 aa, synthetic construct
KYKAKRRNYK

SEQ ID NO: 6 - protein, 10 aa, synthetic construct
KYKARRKNYK

SEQ ID NO: 7 - protein, 10 aa, synthetic construct
KYKARRRNYK

SEQ ID NO: 8 - protein, 10 aa, synthetic construct
KYKARKRNYK

SEQ ID NO: 9 - protein, 10 aa, synthetic construct
KYKAKKKSYK

SEQ ID NO: 10 - protein, 10 aa, synthetic construct
KYKAKKRSYK

SEQ ID NO: 11 - protein, 10 aa, synthetic construct
KYKAKRKSYK

SEQ ID NO: 12 - protein, 10 aa, synthetic construct
KYKARKKSYK

SEQ ID NO: 13 - protein, 10 aa, synthetic construct
KYKAKRRSYK

SEQ ID NO: 14 - protein, 10 aa, synthetic construct
KYKARRKSYK

SEQ ID NO: 15 - protein, 10 aa, synthetic construct
KYKARRRSYK

SEQ ID NO: 16 - protein, 10 aa, synthetic construct
KYKARKRSYK

SEQ ID NO: 17 - protein, 10 aa, synthetic construct
KYRAKKKNYK

SEQ ID NO: 18 - protein, 10 aa, synthetic construct
KYRAKKRNYK

SEQ ID NO: 19 - protein, 10 aa, synthetic construct
KYRAKRKNYK

SEQ ID NO: 20 - protein, 10 aa, synthetic construct
KYRARKKNYK

SEQ ID NO: 21 - protein, 10 aa, synthetic construct
KYRAKRRNYK

SEQ ID NO: 22 - protein, 10 aa, synthetic construct
KYRARRKNYK

SEQ ID NO: 23 - protein, 10 aa, synthetic construct
KYRARRRNYK

SEQ ID NO: 24 - protein, 10 aa, synthetic construct
KYRARKRNYK

SEQ ID NO: 25 - protein, 10 aa, synthetic construct
KYRAKKKSYK

SEQ ID NO: 26 - protein, 10 aa, synthetic construct
KYRAKKRSYK

SEQ ID NO: 27 - protein, 10 aa, synthetic construct
KYRAKRKSYK

SEQ ID NO: 28 - protein, 10 aa, synthetic construct
KYRARKKSYK

SEQ ID NO: 29 - protein, 10 aa, synthetic construct
KYRAKRRSYK

SEQ ID NO: 30 - protein, 10 aa, synthetic construct
KYRARRKSYK

SEQ ID NO: 31 - protein, 10 aa, synthetic construct
KYRARRRSYK

SEQ ID NO: 32 - protein, 10 aa, synthetic construct
KYRARKRSYK

SEQ ID NO: 33 - protein, 10 aa, synthetic construct
KYAKKKKNYK

SEQ ID NO: 34 - protein, 10 aa, synthetic construct
KYAKKKRNYK

SEQ ID NO: 35 - protein, 10 aa, synthetic construct
KYAKKRKNYK

SEQ ID NO: 36 - protein, 10 aa, synthetic construct
KYAKRKKNYK

SEQ ID NO: 37 - protein, 10 aa, synthetic construct
KYAKKRRNYK

SEQ ID NO: 38 - protein, 10 aa, synthetic construct
KYAKRRKNYK

SEQ ID NO: 39 - protein, 10 aa, synthetic construct
KYAKRRRNYK

SEQ ID NO: 40 - protein, 10 aa, synthetic construct
KYAKRKRNYK

SEQ ID NO: 41 - protein, 10 aa, synthetic construct
KYAKKKKSYK

SEQ ID NO: 42 - protein, 10 aa, synthetic construct
KYAKKKRSYK

SEQ ID NO: 43 - protein, 10 aa, synthetic construct
KYAKKRKSYK

SEQ ID NO: 44 - protein, 10 aa, synthetic construct
KYAKRKKSYK

SEQ ID NO: 45 - protein, 10 aa, synthetic construct
KYAKKRRSYK

SEQ ID NO: 46 - protein, 10 aa, synthetic construct
KYAKRRKSYK

SEQ ID NO: 47 - protein, 10 aa, synthetic construct
KYAKRRRSYK

SEQ ID NO: 48 - protein, 10 aa, synthetic construct
KYAKRKRSYK

SEQ ID NO: 49 - protein, 10 aa, synthetic construct
KYARKKKNYK

SEQ ID NO: 50 - protein, 10 aa, synthetic construct
KYARKKRNYK

SEQ ID NO: 51 - protein, 10 aa, synthetic construct
KYARKRKNYK

SEQ ID NO: 52 - protein, 10 aa, synthetic construct
KYARRKKNYK

SEQ ID NO: 53 - protein, 10 aa, synthetic construct
KYARKRRNYK

SEQ ID NO: 54 - protein, 10 aa, synthetic construct
KYARRRKNYK

SEQ ID NO: 55 - protein, 10 aa, synthetic construct
KYARRRRNYK

SEQ ID NO: 56 - protein, 10 aa, synthetic construct
KYARRKRNYK

SEQ ID NO: 57 - protein, 10 aa, synthetic construct
KYARKKKSYK

SEQ ID NO: 58 - protein, 10 aa, synthetic construct
KYARKKRSYK

SEQ ID NO: 59 - protein, 10 aa, synthetic construct
KYARKRKSYK

SEQ ID NO: 60 - protein, 10 aa, synthetic construct
KYARRKKSYK

SEQ ID NO: 61 - protein, 10 aa, synthetic construct
KYARKRRSYK

SEQ ID NO: 62 - protein, 10 aa, synthetic construct
KYARRRKSYK

SEQ ID NO: 63 - protein, 10 aa, synthetic construct
KYARRRRSYK

SEQ ID NO: 64 - protein, 10 aa, synthetic construct
KYARRKRSYK